European Patent Specification EP 3 274 440 B1, published March 4, 2026. Title: DETECTING ESOPHAGEAL DISORDERS. Applicant: EXACT SCIENCES CORPORATION MAYO FOUNDATION FOR MEDICAL EDUCATION AND RESEARCH. The sequence listing filed with the application follows.

SEQUENCE LISTING (50 sequences)

SEQ ID NO: 1 - DNA, 27 bp, Artificial Sequence
  synthetic
tggcggcggaggtagttttaaagatac

SEQ ID NO: 2 - DNA, 25 bp, Artificial Sequence
  synthetic
tcgatcccgaccgaaaactaacgtc

SEQ ID NO: 3 - DNA, 23 bp, Artificial Sequence
  synthetic
gacgtttgtcgtcgggttcgttc

SEQ ID NO: 4 - DNA, 24 bp, Artificial Sequence
  synthetic
aaaaaccctccgctaccacttcgc

SEQ ID NO: 5 - DNA, 25 bp, Artificial Sequence
  synthetic
ttgagatgttgggtgaaggcgattc

SEQ ID NO: 6 - DNA, 26 bp, Artificial Sequence
  synthetic
cgctaacgcgaaaaaataattcgacg

SEQ ID NO: 7 - DNA, 28 bp, Artificial Sequence
  synthetic
cggttttatttattatgattcgtagcgg

SEQ ID NO: 8 - DNA, 24 bp, Artificial Sequence
  synthetic
cgactaccctaaacaacgcatcgc

SEQ ID NO: 9 - DNA, 17 bp, Artificial Sequence
  synthetic
gcgcgtagcggcgtttc

SEQ ID NO: 10 - DNA, 19 bp, Artificial Sequence
  synthetic
cccatatcgcccgacgtaa

SEQ ID NO: 11 - DNA, 34 bp, Artificial Sequence
  synthetic
ttatatttttcgtttttagtaatttcgcgttagc

SEQ ID NO: 12 - DNA, 23 bp, Artificial Sequence
  synthetic
gaaaacccgccgaaacatttcga

SEQ ID NO: 13 - DNA, 23 bp, Artificial Sequence
  synthetic
gtttaattttcggtttcgtcgtc

SEQ ID NO: 14 - DNA, 18 bp, Artificial Sequence
  synthetic
cgctacgaaacactccga

SEQ ID NO: 15 - DNA, 21 bp, Artificial Sequence
  synthetic
cggttttcgttcgttttttcg

SEQ ID NO: 16 - DNA, 18 bp, Artificial Sequence
  synthetic
ccgccttctacgcgacta

SEQ ID NO: 17 - DNA, 30 bp, Artificial Sequence
  synthetic
ggggcgttgtttaacgtatcgaatagttac

SEQ ID NO: 18 - DNA, 30 bp, Artificial Sequence
  synthetic
gctacaaaccctctacccacctaaatcgac

SEQ ID NO: 19 - DNA, 25 bp, Artificial Sequence
  synthetic
ttttagtaagggtcgtattggacgt

SEQ ID NO: 20 - DNA, 27 bp, Artificial Sequence
  synthetic
caaaaactcgctaacacgaaactcccg

SEQ ID NO: 21 - DNA, 16 bp, Artificial Sequence
  synthetic
gttcgtcgttcgggtc

SEQ ID NO: 22 - DNA, 19 bp, Artificial Sequence
  synthetic
tccttcgctaccgaaaacg

SEQ ID NO: 23 - DNA, 19 bp, Artificial Sequence
  synthetic
gtttcgttacggattcgtc

SEQ ID NO: 24 - DNA, 19 bp, Artificial Sequence
  synthetic
tactcgtaaaaaaacgccg

SEQ ID NO: 25 - DNA, 19 bp, Artificial Sequence
  synthetic
ggttcggttgtcgtagcgc

SEQ ID NO: 26 - DNA, 20 bp, Artificial Sequence
  synthetic
ccgaccgtaatcctcgacga

SEQ ID NO: 27 - DNA, 24 bp, Artificial Sequence
  synthetic
gttaatttcgcgaggtaggcgacg

SEQ ID NO: 28 - DNA, 33 bp, Artificial Sequence
  synthetic
cgtaatacaatactcttatatattaacgccgct

SEQ ID NO: 29 - DNA, 24 bp, Artificial Sequence
  synthetic
tgtggaatcggggtttgtgttcgc

SEQ ID NO: 30 - DNA, 25 bp, Artificial Sequence
  synthetic
cccacccaacacaaaaaatccgacg

SEQ ID NO: 31 - DNA, 24 bp, Artificial Sequence
  synthetic
ggagtttattttgggaagagtcgc

SEQ ID NO: 32 - DNA, 20 bp, Artificial Sequence
  synthetic
ccccgcaatcgaaacaaacg

SEQ ID NO: 33 - DNA, 29 bp, Artificial Sequence
  synthetic
gggtagagaatatatagtgaagagtacgg

SEQ ID NO: 34 - DNA, 27 bp, Artificial Sequence
  synthetic
actaaatcacctcctactactaacgct

SEQ ID NO: 35 - DNA, 19 bp, Artificial Sequence
  synthetic
gcgacgtagtcgtcgttgt

SEQ ID NO: 36 - DNA, 19 bp, Artificial Sequence
  synthetic
ccaacgcgaaaaaaacgcg

SEQ ID NO: 37 - DNA, 25 bp, Artificial Sequence
  synthetic
gtttcgttcgaaaggtaggggttcg

SEQ ID NO: 38 - DNA, 25 bp, Artificial Sequence
  synthetic
cgaatctcccgaaaaataaaacgtt

SEQ ID NO: 39 - DNA, 19 bp, Artificial Sequence
  synthetic
tcggagtcgagtttagcgc

SEQ ID NO: 40 - DNA, 24 bp, Artificial Sequence
  synthetic
cgaaatcgaaaaaacaaaaaccgc

SEQ ID NO: 41 - DNA, 19 bp, Artificial Sequence
  synthetic
gtcgtcgttcgagagggta

SEQ ID NO: 42 - DNA, 22 bp, Artificial Sequence
  synthetic
cgaacaaaaacgaacgaacgaa

SEQ ID NO: 43 - DNA, 20 bp, Artificial Sequence
  synthetic
cgccgaggcggttttttgcg

SEQ ID NO: 44 - DNA, 21 bp, Artificial Sequence
  synthetic
ccacggacggttcgtttatcg

SEQ ID NO: 45 - DNA, 20 bp, Artificial Sequence
  synthetic
cgccgaggcggcgttcgcga

SEQ ID NO: 46 - DNA, 21 bp, Artificial Sequence
  synthetic
ccacggacgatcggtttcgtt

SEQ ID NO: 47 - DNA, 25 bp, Artificial Sequence
  synthetic
tgcgtaggtgatagggaggggttac

SEQ ID NO: 48 - DNA, 25 bp, Artificial Sequence
  synthetic
acaaaacacatcctattaacgcgaa

SEQ ID NO: 49 - DNA, 29 bp, Artificial Sequence
  synthetic
tttttatatttcgggaatttagaaacgtc

SEQ ID NO: 50 - DNA, 29 bp, Artificial Sequence
  synthetic
taaaccgaaattaaaaaaaaaattacgcg